European Patent Specification EP 4 059 948 B1, published September 23, 2026. Title: Bar-coded EV library. Applicant: University of Tokyo. The sequence listing filed with the application follows.

SEQUENCE LISTING (50 sequences)

SEQ ID NO: 1 - RNA, 19 nt, Artificial Sequence
  MS2 binding RNA
acaugaggaucacccaugu

SEQ ID NO: 2 - RNA, 65 nt, Artificial Sequence
  Cas9 binding RNA
cagcauagcaaguuuaaauaaggcuaguccguuaucaacuugaaaaaguggcaccgagucggugc

SEQ ID NO: 3 - RNA, 29 nt, Artificial Sequence
  L7Ae binding RNA
ggguaccgugauccgaaaggugaguaccc

SEQ ID NO: 4 - RNA, 15 nt, Artificial Sequence
  LBAPN binding RNA
gcccugaagaagggc

SEQ ID NO: 5 - RNA, 45 nt, Artificial Sequence
  HuR binding RNA
auuuacccauuuacccauuuacccauuuacccauuuacccauuua

SEQ ID NO: 6 - protein, 364 aa, Artificial Sequence
  CD63-L7Ae
MAVEGGMKCVKFLLYVLLLAFCACAVGLIAVGVGAQLVLSQTIIQGATPGSLLPVVIIAVGVFLFLVAFVGCCGACKENYCLMITFAIFLSLIMLVEVAAAIAGYVFRDKVMSEFNNNFRQQMENYPKNNHTASILDRMQADFKCCGAANYTDWEKIPSMSKNRVPDSCCINVTVGCGINFNEKAIHKEGCVEKIGGWLRKNVLVVAAAALGIAFVEVLGIVFACCLVKSIRSGYEVMEFGGGGSMYVRFEVPEDMQNEALSLLEKVRESGKVKKGTNETTKAVERGLAKLVYIAEDVDPPEIVAHLPLLCEEKNVPYIYVKSKNDLGRAVGIEVPCASAAIINEGELRKELGSLVEKIKGLQK

SEQ ID NO: 7 - protein, 376 aa, Artificial Sequence
  CD63-MS2
MAVEGGMKCVKFLLYVLLLAFCACAVGLIAVGVGAQLVLSQTIIQGATPGSLLPVVIIAVGVFLFLVAFVGCCGACKENYCLMITFAIFLSLIMLVEVAAAIAGYVFRDKVMSEFNNNFRQQMENYPKNNHTASILDRMQADFKCCGAANYTDWEKIPSMSKNRVPDSCCINVTVGCGINFNEKAIHKEGCVEKIGGWLRKNVLVVAAAALGIAFVEVLGIVFACCLVKSIRSGYEVMELGGGGSMASNFTQFVLVDNGGTGDVTVAPSNFANGVAEWISSNSRSQAYKVTCSVRQSSAQKRKYTIKVEVPKVATQTVGGVELPVAAWRSYLNMELTIPIFATNSDCELIVKAMQGLLKDGNPIPSAIAANSGIYA

SEQ ID NO: 8 - protein, 1614 aa, Artificial Sequence
  CD63-dCas9
MAVEGGMKCVKFLLYVLLLAFCACAVGLIAVGVGAQLVLSQTIIQGATPGSLLPVVIIAVGVFLFLVAFVGCCGACKENYCLMITFAIFLSLIMLVEVAAAIAGYVFRDKVMSEFNNNFRQQMENYPKNNHTASILDRMQADFKCCGAANYTDWEKIPSMSKNRVPDSCCINVTVGCGINFNEKAIHKEGCVEKIGGWLRKNVLVVAAAALGIAFVEVLGIVFACCLVKSIRSGYEVMEFGGGGSGTDKKYSIGLAIGTNSVGWAVITDEYKVPSKKFKVLGNTDRHSIKKNLIGALLFDSGETAEATRLKRTARRRYTRRKNRICYLQEIFSNEMAKVDDSFFHRLEESFLVEEDKKHERHPIFGNIVDEVAYHEKYPTIYHLRKKLVDSTDKADLRLIYLALAHMIKFRGHFLIEGDLNPDNSDVDKLFIQLVQTYNQLFEENPINASGVDAKAILSARLSKSRRLENLIAQLPGEKKNGLFGNLIALSLGLTPNFKSNFDLAEDAKLQLSKDTYDDDLDNLLAQIGDQYADLFLAAKNLSDAILLSDILRVNTEITKAPLSASMIKRYDEHHQDLTLLKALVRQQLPEKYKEIFFDQSKNGYAGYIDGGASQEEFYKFIKPILEKMDGTEELLVKLNREDLLRKQRTFDNGSIPHQIHLGELHAILRRQEDFYPFLKDNREKIEKILTFRIPYYVGPLARGNSRFAWMTRKSEETITPWNFEEVVDKGASAQSFIERMTNFDKNLPNEKVLPKHSLLYEYFTVYNELTKVKYVTEGMRKPAFLSGEQKKAIVDLLFKTNRKVTVKQLKEDYFKKIECFDSVEISGVEDRFNASLGTYHDLLKIIKDKDFLDNEENEDILEDIVLTLTLFEDREMIEERLKTYAHLFDDKVMKQLKRRRYTGWGRLSRKLINGIRDKQSGKTILDFLKSDGFANRNFMQLIHDDSLTFKEDIQKAQVSGQGDSLHEHIANLAGSPAIKKGILQTVKVVDELVKVMGRHKPENIVIEMARENQTTQKGQKNSRERMKRIEEGIKELGSQILKEHPVENTQLQNEKLYLYYLQNGRDMYVDQELDINRLSDYDVDHIVPQSFLKDDSIDNKVLTRSDKARGKSDNVPSEEVVKKMKNYWRQLLNAKLITQRKFDNLTKAERGGLSELDKAGFIKRQLVETRQITKHVAQILDSRMNTKYDENDKLIREVKVITLKSKLVSDFRKDFQFYKVREINNYHHAHDAYLNAVVGTALIKKYPKLESEFVYGDYKVYDVRKMIAKSEQEIGKATAKYFFYSNIMNFFKTEITLANGEIRKRPLIETNGETGEIVWDKGRDFATVRKVLSMPQVNIVKKTEVQTGGFSKESILPKRNSDKLIARKKDWDPKKYGGFDSPTVAYSVLVVAKVEKGKSKKLKSVKELLGITIMERSSFEKNPIDFLEAKGYKEVKKDLIIKLPKYSLFELENGRKRMLASAGELQKGNELALPSKYVNFLYLASHYEKLKGSPEDNEQKQLFVEQHKHYLDEIIEQISEFSKRVILADANLDKVLSAYNKHRDKPIREQAENIIHLFTLTNLGAPAAFKYFDTTIDRKRYTSTKEVLDATLIHQSITGLYETRIDLSQLGGD

SEQ ID NO: 9 - protein, 1605 aa, Artificial Sequence
  CD9-dCas9
MPVKGGTKCIKYLLFGFNFIFWLAGIAVLAIGLWLRFDSQTKSIFEQETNNNNSSFYTGVYILIGAGALMMLVGFLGCCGAVQESQCMLGLFFGFLLVIFAIEIAAAIWGYSHKDEVIKEVQEFYKDTYNKLKTKDEPQRETLKAIHYALNCCGLAGGVEQFISDICPKKDVLETFTVKSCPDAIKEVFDNKFHIIGAVGIGIAVVMIFGMIFSMILCCAIRRNREMVLEFGGGGSGTDKKYSIGLAIGTNSVGWAVITDEYKVPSKKFKVLGNTDRHSIKKNLIGALLFDSGETAEATRLKRTARRRYTRRKNRICYLQEIFSNEMAKVDDSFFHRLEESFLVEEDKKHERHPIFGNIVDEVAYHEKYPTIYHLRKKLVDSTDKADLRLIYLALAHMIKFRGHFLIEGDLNPDNSDVDKLFIQLVQTYNQLFEENPINASGVDAKAILSARLSKSRRLENLIAQLPGEKKNGLFGNLIALSLGLTPNFKSNFDLAEDAKLQLSKDTYDDDLDNLLAQIGDQYADLFLAAKNLSDAILLSDILRVNTEITKAPLSASMIKRYDEHHQDLTLLKALVRQQLPEKYKEIFFDQSKNGYAGYIDGGASQEEFYKFIKPILEKMDGTEELLVKLNREDLLRKQRTFDNGSIPHQIHLGELHAILRRQEDFYPFLKDNREKIEKILTFRIPYYVGPLARGNSRFAWMTRKSEETITPWNFEEVVDKGASAQSFIERMTNFDKNLPNEKVLPKHSLLYEYFTVYNELTKVKYVTEGMRKPAFLSGEQKKAIVDLLFKTNRKVTVKQLKEDYFKKIECFDSVEISGVEDRFNASLGTYHDLLKIIKDKDFLDNEENEDILEDIVLTLTLFEDREMIEERLKTYAHLFDDKVMKQLKRRRYTGWGRLSRKLINGIRDKQSGKTILDFLKSDGFANRNFMQLIHDDSLTFKEDIQKAQVSGQGDSLHEHIANLAGSPAIKKGILQTVKVVDELVKVMGRHKPENIVIEMARENQTTQKGQKNSRERMKRIEEGIKELGSQILKEHPVENTQLQNEKLYLYYLQNGRDMYVDQELDINRLSDYDVDHIVPQSFLKDDSIDNKVLTRSDKARGKSDNVPSEEVVKKMKNYWRQLLNAKLITQRKFDNLTKAERGGLSELDKAGFIKRQLVETRQITKHVAQILDSRMNTKYDENDKLIREVKVITLKSKLVSDFRKDFQFYKVREINNYHHAHDAYLNAVVGTALIKKYPKLESEFVYGDYKVYDVRKMIAKSEQEIGKATAKYFFYSNIMNFFKTEITLANGEIRKRPLIETNGETGEIVWDKGRDFATVRKVLSMPQVNIVKKTEVQTGGFSKESILPKRNSDKLIARKKDWDPKKYGGFDSPTVAYSVLVVAKVEKGKSKKLKSVKELLGITIMERSSFEKNPIDFLEAKGYKEVKKDLIIKLPKYSLFELENGRKRMLASAGELQKGNELALPSKYVNFLYLASHYEKLKGSPEDNEQKQLFVEQHKHYLDEIIEQISEFSKRVILADANLDKVLSAYNKHRDKPIREQAENIIHLFTLTNLGAPAAFKYFDTTIDRKRYTSTKEVLDATLIHQSITGLYETRIDLSQLGGD

SEQ ID NO: 10 - protein, 1392 aa, Artificial Sequence
  Cas9(SpCas9-NLS-FLAG)
MDKKYSIGLDIGTNSVGWAVITDEYKVPSKKFKVLGNTDRHSIKKNLIGALLFDSGETAEATRLKRTARRRYTRRKNRICYLQEIFSNEMAKVDDSFFHRLEESFLVEEDKKHERHPIFGNIVDEVAYHEKYPTIYHLRKKLVDSTDKADLRLIYLALAHMIKFRGHFLIEGDLNPDNSDVDKLFIQLVQTYNQLFEENPINASGVDAKAILSARLSKSRRLENLIAQLPGEKKNGLFGNLIALSLGLTPNFKSNFDLAEDAKLQLSKDTYDDDLDNLLAQIGDQYADLFLAAKNLSDAILLSDILRVNTEITKAPLSASMIKRYDEHHQDLTLLKALVRQQLPEKYKEIFFDQSKNGYAGYIDGGASQEEFYKFIKPILEKMDGTEELLVKLNREDLLRKQRTFDNGSIPHQIHLGELHAILRRQEDFYPFLKDNREKIEKILTFRIPYYVGPLARGNSRFAWMTRKSEETITPWNFEEVVDKGASAQSFIERMTNFDKNLPNEKVLPKHSLLYEYFTVYNELTKVKYVTEGMRKPAFLSGEQKKAIVDLLFKTNRKVTVKQLKEDYFKKIECFDSVEISGVEDRFNASLGTYHDLLKIIKDKDFLDNEENEDILEDIVLTLTLFEDREMIEERLKTYAHLFDDKVMKQLKRRRYTGWGRLSRKLINGIRDKQSGKTILDFLKSDGFANRNFMQLIHDDSLTFKEDIQKAQVSGQGDSLHEHIANLAGSPAIKKGILQTVKVVDELVKVMGRHKPENIVIEMARENQTTQKGQKNSRERMKRIEEGIKELGSQILKEHPVENTQLQNEKLYLYYLQNGRDMYVDQELDINRLSDYDVDHIVPQSFLKDDSIDNKVLTRSDKNRGKSDNVPSEEVVKKMKNYWRQLLNAKLITQRKFDNLTKAERGGLSELDKAGFIKRQLVETRQITKHVAQILDSRMNTKYDENDKLIREVKVITLKSKLVSDFRKDFQFYKVREINNYHHAHDAYLNAVVGTALIKKYPKLESEFVYGDYKVYDVRKMIAKSEQEIGKATAKYFFYSNIMNFFKTEITLANGEIRKRPLIETNGETGEIVWDKGRDFATVRKVLSMPQVNIVKKTEVQTGGFSKESILPKRNSDKLIARKKDWDPKKYGGFDSPTVAYSVLVVAKVEKGKSKKLKSVKELLGITIMERSSFEKNPIDFLEAKGYKEVKKDLIIKLPKYSLFELENGRKRMLASAGELQKGNELALPSKYVNFLYLASHYEKLKGSPEDNEQKQLFVEQHKHYLDEIIEQISEFSKRVILADANLDKVLSAYNKHRDKPIREQAENIIHLFTLTNLGAPAAFKYFDTTIDRKRYTSTKEVLDATLIHQSITGLYETRIDLSQLGGDKRPAATKKAGQAKKKKDYKDDDDK

SEQ ID NO: 11 - protein, 1932 aa, Artificial Sequence
  dCas9-VPR
MDKKYSIGLAIGTNSVGWAVITDEYKVPSKKFKVLGNTDRHSIKKNLIGALLFDSGETAEATRLKRTARRRYTRRKNRICYLQEIFSNEMAKVDDSFFHRLEESFLVEEDKKHERHPIFGNIVDEVAYHEKYPTIYHLRKKLVDSTDKADLRLIYLALAHMIKFRGHFLIEGDLNPDNSDVDKLFIQLVQTYNQLFEENPINASGVDAKAILSARLSKSRRLENLIAQLPGEKKNGLFGNLIALSLGLTPNFKSNFDLAEDAKLQLSKDTYDDDLDNLLAQIGDQYADLFLAAKNLSDAILLSDILRVNTEITKAPLSASMIKRYDEHHQDLTLLKALVRQQLPEKYKEIFFDQSKNGYAGYIDGGASQEEFYKFIKPILEKMDGTEELLVKLNREDLLRKQRTFDNGSIPHQIHLGELHAILRRQEDFYPFLKDNREKIEKILTFRIPYYVGPLARGNSRFAWMTRKSEETITPWNFEEVVDKGASAQSFIERMTNFDKNLPNEKVLPKHSLLYEYFTVYNELTKVKYVTEGMRKPAFLSGEQKKAIVDLLFKTNRKVTVKQLKEDYFKKIECFDSVEISGVEDRFNASLGTYHDLLKIIKDKDFLDNEENEDILEDIVLTLTLFEDREMIEERLKTYAHLFDDKVMKQLKRRRYTGWGRLSRKLINGIRDKQSGKTILDFLKSDGFANRNFMQLIHDDSLTFKEDIQKAQVSGQGDSLHEHIANLAGSPAIKKGILQTVKVVDELVKVMGRHKPENIVIEMARENQTTQKGQKNSRERMKRIEEGIKELGSQILKEHPVENTQLQNEKLYLYYLQNGRDMYVDQELDINRLSDYDVAAIVPQSFLKDDSIDNKVLTRSDKARGKSDNVPSEEVVKKMKNYWRQLLNAKLITQRKFDNLTKAERGGLSELDKAGFIKRQLVETRQITKHVAQILDSRMNTKYDENDKLIREVKVITLKSKLVSDFRKDFQFYKVREINNYHHAHDAYLNAVVGTALIKKYPKLESEFVYGDYKVYDVRKMIAKSEQEIGKATAKYFFYSNIMNFFKTEITLANGEIRKRPLIETNGETGEIVWDKGRDFATVRKVLSMPQVNIVKKTEVQTGGFSKESILPKRNSDKLIARKKDWDPKKYGGFDSPTVAYSVLVVAKVEKGKSKKLKSVKELLGITIMERSSFEKNPIDFLEAKGYKEVKKDLIIKLPKYSLFELENGRKRMLASAGELQKGNELALPSKYVNFLYLASHYEKLKGSPEDNEQKQLFVEQHKHYLDEIIEQISEFSKRVILADANLDKVLSAYNKHRDKPIREQAENIIHLFTLTNLGAPAAFKYFDTTIDRKRYTSTKEVLDATLIHQSITGLYETRIDLSQLGGDSRADPKKKRKVSPGIRRLDALISTSLYKKAGYKEASGSGRADALDDFDLDMLGSDALDDFDLDMLGSDALDDFDLDMLGSDALDDFDLDMLINSRSSGSPKKKRKVGSQYLPDTDDRHRIEEKRKRTYETFKSIMKKSPFSGPTDPRPPPRRIAVPSRSSASVPKPAPQPYPFTSSLSTINYDEFPTMVFPSGQISQASALAPAPPQVLPQAPAPAPAPAMVSALAQAPAPVPVLAPGPPQAVAPPAPKPTQAGEGTLSEALLQLQFDDEDLGALLGNSTDPAVFTDLASVDNSEFQQLLNQGIPVAPHTTEPMLMEYPEAITRLVTGAQRPPDPAPAPLGAPGLPNGLLSGDEDFSSIADMDFSALLGSGSGSRDSREGMFLPKPEAGSAISDVFEGREVCQPKRIRPFHPPGSPWANRPLPASLAPTPTGPVHEPVGSLTPAPVPQPLDPAPAVTPEASHLLEDPDEETSQAVKALREMADTVIPQKEEAAICGQMDLSHPPPRGHLDELTTTLESMTEDLNLDSPLTPELNEILDTFLNDECLLHAMHISTGLSIFDTSLF

SEQ ID NO: 12 - DNA, 149 bp, Artificial Sequence
  C/D box
gctaagccagggcgtgatgcgaaagctgacccctgcagggcctagcaagttaaaataaggctagtccgttatcaacttggccagggcgtgatgcgaaagctgacccctgcagggccaagtggcaccgagtcggtgctttttttctcgag

SEQ ID NO: 13 - DNA, 28 bp, Artificial Sequence
  LNA
  ribonucleotide (26)..(27)
  modified_base (28)..(28): 2'-4' bridged nucleic acid
aagcagtggtatcaacgcagagtacggg

SEQ ID NO: 14 - DNA, 21 bp, Artificial Sequence
  RT primer
aaagcaccgactcggtgccac

SEQ ID NO: 15 - DNA, 21 bp, Artificial Sequence
  RT primer
attttgcataaaggcaagtgg

SEQ ID NO: 16 - DNA, 26 bp, Artificial Sequence
  RT primer
tttttcaagttgataacggactagcc

SEQ ID NO: 17 - DNA, 17 bp, Artificial Sequence
  for backbone_gRNA
ggtcttcgagaagacct

SEQ ID NO: 18 - DNA, 20 bp, Artificial Sequence
  for CD274_gRNA
ctatacacagctttattcct

SEQ ID NO: 19 - DNA, 20 bp, Artificial Sequence
  for CD274_gRNA
ctgaccttcggtgaaatcgg

SEQ ID NO: 20 - DNA, 20 bp, Artificial Sequence
  for CD47_gRNA
caggacgtgacctggaagcg

SEQ ID NO: 21 - DNA, 20 bp, Artificial Sequence
  for CD47_gRNA
gcgtgccaccgccctggagc

SEQ ID NO: 22 - DNA, 20 bp, Artificial Sequence
  for CD55_gRNA
aaacggggtgtaaacgggag

SEQ ID NO: 23 - DNA, 20 bp, Artificial Sequence
  for CD55_gRNA
gaactcacgtgcgggcagca

SEQ ID NO: 24 - DNA, 20 bp, Artificial Sequence
  for CD59_gRNA
accccagggaactgaaagtt

SEQ ID NO: 25 - DNA, 20 bp, Artificial Sequence
  for CD59_gRNA
caggttctgagaaggccggg

SEQ ID NO: 26 - DNA, 20 bp, Artificial Sequence
  for CD81_gRNA
ccgccagggcgcgcagccga

SEQ ID NO: 27 - DNA, 20 bp, Artificial Sequence
  for ICAM1_gRNA
cagtttaccgctttgtgaaa

SEQ ID NO: 28 - DNA, 20 bp, Artificial Sequence
  for ICAM1_gRNA
cctccctctccagcttacgc

SEQ ID NO: 29 - DNA, 20 bp, Artificial Sequence
  for IL1B_gRNA
aaaaacagcgagggagaaac

SEQ ID NO: 30 - DNA, 20 bp, Artificial Sequence
  for ITGAL_gRNA
gacagtctccactgctgtca

SEQ ID NO: 31 - DNA, 20 bp, Artificial Sequence
  for ITGAL_gRNA
ggctctgtaaagctcagcag

SEQ ID NO: 32 - DNA, 20 bp, Artificial Sequence
  for LRP1_gRNA
atcggcgcatgcgcactcac

SEQ ID NO: 33 - DNA, 20 bp, Artificial Sequence
  for LRP1_gRNA
ctgcccgggggagggcgacg

SEQ ID NO: 34 - protein, 450 aa, Artificial Sequence
  4mer-random peptide fused Lamp2b
  MISC_FEATURE (38)..(42): random amino acid
  MISC_FEATURE (38)..(42): random peptide
  MISC_FEATURE (39)..(42): random amino acid
MVCFRLFPVPGSGLVLVCLVLGAVRSYAGNSTMGSGCGXXXXGGCGGSGSGSGGSSLELNLTDSENATCLYAKWQMNFTVRYETTNKTYKTVTISDHGTVTYNGSICGDDQNGPKIAVQFGPGFSWIANFTKAASTYSIDSVSFSYNTGDNTTFPDAEDKGILTVDELLAIRIPLNDLFRCNSLSTLEKNDVVQHYWDVLVQAFVQNGTVSTNEFLCDKDKTSTVAPTIHTTVPSPTTTPTPKEKPEAGTYSVNNGNDTCLLATMGLQLNITQDKVASVININPNTTHSTGSCRSHTALLRLNSSTIKYLDFVFAVKNENRFYLKEVNISMYLVNGSVFSIANNNLSYWDAPLGSSYMCNKEQTVSVSGAFQINTFDLRVQPFNVTQGKYSTAQECSLDDDTILIPIIVGAGLSGLIIVIVIAYVIGRRKSYAGYQTLGSGYPYDVPDYA

SEQ ID NO: 35 - DNA, 20 bp, Artificial Sequence
  for ABCG4_gRNA
gctccgtggggacaagtccc

SEQ ID NO: 36 - DNA, 20 bp, Artificial Sequence
  for IL1RL2_gRNA
ggcatggaagtggcatgaca

SEQ ID NO: 37 - DNA, 20 bp, Artificial Sequence
  for TMEM14B_gRNA
gcacgcgccctgcatcccgg

SEQ ID NO: 38 - DNA, 20 bp, Artificial Sequence
  for SLAMF1_gRNA
gaacccgcttcctgtatcac

SEQ ID NO: 39 - DNA, 20 bp, Artificial Sequence
  for SLC28A1_gRNA
ggggaccccaacacggtctc

SEQ ID NO: 40 - DNA, 20 bp, Artificial Sequence
  for SLC39A8_gRNA
gaccgccggccttccctccg

SEQ ID NO: 41 - DNA, 20 bp, Artificial Sequence
  for OR1N1_gRNA
gtccccttccaataaggtca

SEQ ID NO: 42 - DNA, 20 bp, Artificial Sequence
  for FAM155A_gRNA
ggggaggcggcgtcagcagt

SEQ ID NO: 43 - DNA, 20 bp, Artificial Sequence
  for MPZL1_gRNA
gcggggccgaggcgcctggg

SEQ ID NO: 44 - DNA, 20 bp, Artificial Sequence
  for OR5K1_gRNA
gtggtgcatgccccattcat

SEQ ID NO: 45 - DNA, 20 bp, Artificial Sequence
  for LPHN2_gRNA
gaatgttcataaaaatcgga

SEQ ID NO: 46 - DNA, 20 bp, Artificial Sequence
  for SLC47A2_gRNA
gggctaccatggcaacttgt

SEQ ID NO: 47 - DNA, 20 bp, Artificial Sequence
  for OR1J2_gRNA
gctccccacagacccccgat

SEQ ID NO: 48 - DNA, 20 bp, Artificial Sequence
  for LRIT3_gRNA
ggtaatctgctgttactaaa

SEQ ID NO: 49 - DNA, 20 bp, Artificial Sequence
  for PODXL_gRNA
ggccgctggcgggctcctgg

SEQ ID NO: 50 - DNA, 20 bp, Artificial Sequence
  for TSPAN2_gRNA
gggggcgcgtggaccccaag